European Patent Application EP 4 564 005 A1, published June 4, 2025. Title: IN VITRO METHOD FOR DIAGNOSING OR SCREENING CHRONIC INFLAMMATORY DISEASES. Applicant: AIRBIOMETRICS ADVANCED. Application EP. The sequence listing filed with the application follows.

SEQUENCE LISTING (8 sequences)

SEQ ID NO: 1 - DNA, 21 bp, synthetic construct
  source 1..21: mol_type = other DNA
tttttgctgtgagtcccggag

SEQ ID NO: 2 - DNA, 21 bp, synthetic construct
  source 1..21: mol_type = other DNA
tttttgctgtgagtcccggag

SEQ ID NO: 3 - DNA, 20 bp, synthetic construct
  source 1..20: mol_type = other DNA
agtggccaagatcacagtgg

SEQ ID NO: 4 - DNA, 20 bp, synthetic construct
  source 1..20: mol_type = other DNA
gcctggcctcctgattagtg

SEQ ID NO: 5 - DNA, 21 bp, synthetic construct
  source 1..21: mol_type = other DNA
tccaagttccataccccatga

SEQ ID NO: 6 - DNA, 21 bp, synthetic construct
  source 1..21: mol_type = other DNA
caaaatgcagatgaggcaaag

SEQ ID NO: 7 - DNA, 20 bp, synthetic construct
  source 1..20: mol_type = other DNA
cggctaccacatccaaggaa

SEQ ID NO: 8 - DNA, 18 bp, synthetic construct
  source 1..18: mol_type = other DNA
gtcggaattaccgcggct